European Patent Application EP 4 474 474 A2, published December 11, 2024. Title: METHODS AND COMPOSITIONS FOR THE TREATMENT OF OSTEOPETROSIS. Applicant: MEMORIAL SLOAN KETTERING CANCER CENTER. The sequence listing filed with the application follows.

SEQUENCE LISTING (38 sequences)

SEQ ID NO: 1 - DNA, 20 bp, synthetic construct
  misc_feature 1..20: note = Description of Artificial Sequence: Synthetic primer
  source 1..20: mol_type = other DNA
tctctgcccagagtcatcct

SEQ ID NO: 2 - DNA, 20 bp, synthetic construct
  misc_feature 1..20: note = Description of Artificial Sequence: Synthetic primer
  source 1..20: mol_type = other DNA
ctctgacagatgccaggaca

SEQ ID NO: 3 - DNA, 20 bp, synthetic construct
  misc_feature 1..20: note = Description of Artificial Sequence: Synthetic primer
  source 1..20: mol_type = other DNA
tcgaagcttgcatgcctgca

SEQ ID NO: 4 - DNA, 20 bp, synthetic construct
  misc_feature 1..20: note = Description of Artificial Sequence: Synthetic primer
  source 1..20: mol_type = other DNA
tctctgcccagagtcatcct

SEQ ID NO: 5 - DNA, 18 bp, synthetic construct
  misc_feature 1..18: note = Description of Artificial Sequence: Synthetic primer
  source 1..18: mol_type = other DNA
tcattccagaaccagagc

SEQ ID NO: 6 - DNA, 18 bp, synthetic construct
  misc_feature 1..18: note = Description of Artificial Sequence: Synthetic primer
  source 1..18: mol_type = other DNA
gatcgtgttggggaagcc

SEQ ID NO: 7 - DNA, 20 bp, synthetic construct
  misc_feature 1..20: note = Description of Artificial Sequence: Synthetic primer
  source 1..20: mol_type = other DNA
gccaccatgtgtccgtgctt

SEQ ID NO: 8 - DNA, 20 bp, synthetic construct
  misc_feature 1..20: note = Description of Artificial Sequence: Synthetic primer
  source 1..20: mol_type = other DNA
acccagagcccccacagata

SEQ ID NO: 9 - DNA, 21 bp, synthetic construct
  misc_feature 1..21: note = Description of Artificial Sequence: Synthetic primer
  source 1..21: mol_type = other DNA
ggtggatgtggaatgtgtgcg

SEQ ID NO: 10 - DNA, 21 bp, synthetic construct
  misc_feature 1..21: note = Description of Artificial Sequence: Synthetic primer
  source 1..21: mol_type = other DNA
cgtttcttgtggtcagggtgc

SEQ ID NO: 11 - DNA, 20 bp, synthetic construct
  misc_feature 1..20: note = Description of Artificial Sequence: Synthetic primer
  source 1..20: mol_type = other DNA
acggagtccaggcaacttcc

SEQ ID NO: 12 - DNA, 20 bp, synthetic construct
  misc_feature 1..20: note = Description of Artificial Sequence: Synthetic primer
  source 1..20: mol_type = other DNA
gaagcatgtttagctggccc

SEQ ID NO: 13 - DNA, 21 bp, synthetic construct
  misc_feature 1..21: note = Description of Artificial Sequence: Synthetic primer
  source 1..21: mol_type = other DNA
ccatgcgtcgcaaggtggaac

SEQ ID NO: 14 - DNA, 20 bp, synthetic construct
  misc_feature 1..20: note = Description of Artificial Sequence: Synthetic primer
  source 1..20: mol_type = other DNA
gtgcttcggcgatgtggtaa

SEQ ID NO: 15 - DNA, 21 bp, synthetic construct
  misc_feature 1..21: note = Description of Artificial Sequence: Synthetic primer
  source 1..21: mol_type = other DNA
ccatgcgtcgcaaggtggaac

SEQ ID NO: 16 - DNA, 22 bp, synthetic construct
  misc_feature 1..22: note = Description of Artificial Sequence: Synthetic primer
  source 1..22: mol_type = other DNA
tggccgcttttctggattcatc

SEQ ID NO: 17 - DNA, 26 bp, synthetic construct
  misc_feature 1..26: note = Description of Artificial Sequence: Synthetic primer
  source 1..26: mol_type = other DNA
gcctgcattaccggtcgatgcaacga

SEQ ID NO: 18 - DNA, 26 bp, synthetic construct
  misc_feature 1..26: note = Description of Artificial Sequence: Synthetic primer
  source 1..26: mol_type = other DNA
aatggtgttgccgcgccatctgccac

SEQ ID NO: 19 - DNA, 20 bp, synthetic construct
  misc_feature 1..20: note = Description of Artificial Sequence: Synthetic primer
  source 1..20: mol_type = other DNA
aagtcgctctgagttgttat

SEQ ID NO: 20 - DNA, 21 bp, synthetic construct
  misc_feature 1..21: note = Description of Artificial Sequence: Synthetic primer
  source 1..21: mol_type = other DNA
ggagcgggagaaatggatatg

SEQ ID NO: 21 - DNA, 20 bp, synthetic construct
  misc_feature 1..20: note = Description of Artificial Sequence: Synthetic primer
  source 1..20: mol_type = other DNA
aagtcgctctgagttgttat

SEQ ID NO: 22 - DNA, 21 bp, synthetic construct
  misc_feature 1..21: note = Description of Artificial Sequence: Synthetic primer
  source 1..21: mol_type = other DNA
gcgaagagtttgtcctcaacc

SEQ ID NO: 23 - DNA, 20 bp, synthetic construct
  misc_feature 1..20: note = Description of Artificial Sequence: Synthetic primer
  source 1..20: mol_type = other DNA
aagggagctgcagtggagta

SEQ ID NO: 24 - DNA, 20 bp, synthetic construct
  misc_feature 1..20: note = Description of Artificial Sequence: Synthetic primer
  source 1..20: mol_type = other DNA
ccgaaaatctgtgggaagtc

SEQ ID NO: 25 - DNA, 20 bp, synthetic construct
  misc_feature 1..20: note = Description of Artificial Sequence: Synthetic primer
  source 1..20: mol_type = other DNA
ggcattaaagcagcgtatcc

SEQ ID NO: 26 - DNA, 19 bp, synthetic construct
  misc_feature 1..19: note = Description of Artificial Sequence: Synthetic primer
  source 1..19: mol_type = other DNA
ctgttcctgtacggcatgg

SEQ ID NO: 27 - DNA, 25 bp, synthetic construct
  misc_feature 1..25: note = Description of Artificial Sequence: Synthetic primer
  source 1..25: mol_type = other DNA
agtgtgcctggcatgtgcagacctt

SEQ ID NO: 28 - DNA, 25 bp, synthetic construct
  misc_feature 1..25: note = Description of Artificial Sequence: Synthetic primer
  source 1..25: mol_type = other DNA
ctggtggttgttctcctggtgtcat

SEQ ID NO: 29 - DNA, 25 bp, synthetic construct
  misc_feature 1..25: note = Description of Artificial Sequence: Synthetic primer
  source 1..25: mol_type = other DNA
agtgtgcctggcatgtgcagacctt

SEQ ID NO: 30 - DNA, 25 bp, synthetic construct
  misc_feature 1..25: note = Description of Artificial Sequence: Synthetic primer
  source 1..25: mol_type = other DNA
ggcagaactcggatgcacagattgg

SEQ ID NO: 31 - DNA, 22 bp, synthetic construct
  misc_feature 1..22: note = Description of Artificial Sequence: Synthetic primer
  source 1..22: mol_type = other DNA
tgaagggtgacatcatcgtggt

SEQ ID NO: 32 - DNA, 18 bp, synthetic construct
  misc_feature 1..18: note = Description of Artificial Sequence: Synthetic primer
  source 1..18: mol_type = other DNA
aataggggtggggtgata

SEQ ID NO: 33 - DNA, 20 bp, synthetic construct
  misc_feature 1..20: note = Description of Artificial Sequence: Synthetic primer
  source 1..20: mol_type = other DNA
acttctccatggtagcctcc

SEQ ID NO: 34 - DNA, 18 bp, synthetic construct
  misc_feature 1..18: note = Description of Artificial Sequence: Synthetic primer
  source 1..18: mol_type = other DNA
aataggggtggggtgata

SEQ ID NO: 35 - DNA, 22 bp, synthetic construct
  misc_feature 1..22: note = Description of Artificial Sequence: Synthetic primer
  source 1..22: mol_type = other DNA
aacctgaggatgtgagggacta

SEQ ID NO: 36 - DNA, 22 bp, synthetic construct
  misc_feature 1..22: note = Description of Artificial Sequence: Synthetic primer
  source 1..22: mol_type = other DNA
gtcaaagtcagtgcgttcaaag

SEQ ID NO: 37 - DNA, 26 bp, synthetic construct
  misc_feature 1..26: note = Description of Artificial Sequence: Synthetic primer
  source 1..26: mol_type = other DNA
gcctgcattaccggtcgatgcaacga

SEQ ID NO: 38 - DNA, 26 bp, synthetic construct
  misc_feature 1..26: note = Description of Artificial Sequence: Synthetic primer
  source 1..26: mol_type = other DNA
aatggtgttgccgcgccatctgccac